European Patent Specification EP 3 810 645 B1, published August 12, 2026. Title: CHIMERIC TRANSMEMBRANE PROTEINS AND USES THEREOF. Applicant: KITE PHARMA, INC. The sequence listing filed with the application follows.

SEQUENCE LISTING (111 sequences)

SEQ ID NO: 1 - protein, 25 aa, Homo sapiens
PILLTISILSFFSVALLVILACVLW

SEQ ID NO: 2 - protein, 25 aa, Artificial Sequence
  source: /note="Description of Artificial Sequence: Synthetic IL7RA EKA sequence"
PILLTISILSFFSVEKAVILACVLW

SEQ ID NO: 3 - DNA, 75 bp, Artificial Sequence
  source: /note="Description of Artificial Sequence: Synthetic IL7RA EKA sequence"
cccatcctgctgaccatcagcatcctgagcttcttcagcgtggagaaggtggtgatcctggcctgcgtgctgtgg

SEQ ID NO: 4 - protein, 25 aa, Artificial Sequence
  source: /note="Description of Artificial Sequence: Synthetic IL7RA EKV sequence"
PILLTISILSFFSVEKVVILACVLW

SEQ ID NO: 5 - DNA, 75 bp, Artificial Sequence; identical to SEQ ID NO: 3
  source: /note="Description of Artificial Sequence: Synthetic IL7RA EKV sequence"

SEQ ID NO: 6 - protein, 28 aa, Artificial Sequence
  source: /note="Description of Artificial Sequence: Synthetic IL7RA CPT insert sequence"
PILLTCPTISILSFFSVALLVILACVLW

SEQ ID NO: 7 - DNA, 84 bp, Artificial Sequence
  source: /note="Description of Artificial Sequence: Synthetic IL7RA CPT insert sequence"
cccatcctgctgacctgccccaccatcagcatcctgagcttcttcagcgtggccctgctggtgatcctggcctgcgtgctgtgg

SEQ ID NO: 8 - protein, 29 aa, Artificial Sequence
  source: /note="Description of Artificial Sequence: Synthetic IL7RA PPCL insert sequence"
PILLPPCLTISILSFFSVALLVILACVLW

SEQ ID NO: 9 - DNA, 87 bp, Artificial Sequence
  source: /note="Description of Artificial Sequence: Synthetic IL7RA PPCL insert sequence"
cccatcctgctgccaccctgtttaaccatcagcatcctgagcttcttcagcgtggccctgctggtgatcctggcctgcgtgctgtgg

SEQ ID NO: 10 - protein, 22 aa, Homo sapiens
MLLLVTSLLLCELPHPAFLLIP

SEQ ID NO: 11 - protein, 220 aa, Homo sapiens
GESGYAQNGDLEDAELDDYSFSCYSQLEVNGSQHSLTCAFEDPDVNITNLEFEICGALVEVKCLNFRKLQEIYFIETKKFLLIGKSNICVKVGEKSLTCKKIDLTTIVKPEAPFDLSVVYREGANDFVVTFNTSHLQKKYVKVLMHDVAYRQEKDENKWTHVNLSSTKLTLLQRKLQPAAMYEIKVRSIPDHYFKGFWSEWSPSYYFRTPEINNSSGEMD

SEQ ID NO: 12 - DNA, 660 bp, Homo sapiens
ggcgagagcggctacgcccagaacggcgacctggaggacgccgagctggacgactacagcttcagctgctacagccagctggaggtgaacggcagccagcacagcctgacctgcgccttcgaggaccccgacgtgaacatcaccaacctggagttcgagatctgcggcgccctggtggaggtgaagtgcctgaacttcaggaagctgcaggagatctacttcatcgagaccaagaagttcctgctgatcggcaagagcaacatctgcgtgaaggtgggcgagaagagcctgacctgcaagaagatcgacctgaccaccatcgtgaagcccgaggcccccttcgacctgagcgtggtgtacagggagggcgccaacgacttcgtggtgaccttcaacaccagccacctgcagaagaagtacgtgaaggtgctgatgcacgacgtggcctacaggcaggagaaggacgagaacaagtggacccacgtgaacctgagcagcaccaagctgaccctgctgcagaggaagctgcagcccgccgccatgtacgagatcaaggtgaggagcatccccgaccactacttcaagggcttctggagcgagtggagccccagctactacttcaggacccccgagatcaacaacagcagcggcgagatggac

SEQ ID NO: 13 - protein, 219 aa, Mus musculus
ESGNAQDGDLEDADADDHSFWCHSQLEVDGSQHLLTCAFNDSDINTANLEFQICGALLRVKCLTLNKLQDIYFIKTSEFLLIGSSNICVKLGQKNLTCKNMAINTIVKAEAPSDLKVVYRKEANDFLVTFNAPHLKKKYLKKVKHDVAYRPARGESNWTHVSLFHTRTTIPQRKLRPKAMYEIKVRSIPHNDYFKGFWSEWSPSSTFETPEPKNQGGWD

SEQ ID NO: 14 - DNA, 657 bp, Mus musculus
gaaagtggaaatgcccaggatggagacctagaagatgcagacgcggacgatcactccttctggtgccacagccagttggaagtggatggaagtcaacatttattgacttgtgcttttaatgactcagacatcaacacagctaatctggaatttcaaatatgtggggctcttttacgagtgaaatgcctaactcttaacaagctgcaagatatatattttataaagacatcagaattcttactgattggtagcagcaatatatgtgtgaagcttggacaaaagaatttaacttgcaaaaatatggctataaacacaatagttaaagccgaggctccctctgacctgaaagtcgtttatcgcaaagaagcaaatgattttttggtgacatttaatgcacctcacttgaaaaagaaatatttaaaaaaagtaaagcatgatgtggcctaccgcccagcaaggggtgaaagcaactggacgcatgtatctttattccacacaagaacaacaatcccacagagaaaactacgaccaaaagcaatgtatgaaatcaaagtccgatccattccccataacgattacttcaaaggcttctggagcgagtggagtccaagttctaccttcgaaactccagaacccaagaatcaaggaggatgggat

SEQ ID NO: 15 - protein, 219 aa, Mus musculus; identical to SEQ ID NO: 13

SEQ ID NO: 16 - DNA, 657 bp, Mus musculus; identical to SEQ ID NO: 14

SEQ ID NO: 17 - protein, 535 aa, Artificial Sequence
  source: /note="Description of Artificial Sequence: Synthetic Exemplary chimeric transmembrane protein sequence"
NWVNVISDLKKIEDLIQSMHIDATLYTESDVHPSCKVTAMKCFLLELQVISLESGDASIHDTVENLIILANNSLSSNGNVTESGCKECEELEEKNIKEFLQSFVHIVQMFINTSSGGGSGGGGSGGGGSGGGGSGGGSLQITCPPPMSVEHADIWVKSYSLYSRERYICNSGFKRKAGTSSLTECVLNKATNVAHWTTPSLKCIRDPALVHQRPAPPSTVTTAGVTPQPESLSPSGKEPAASSPSSNNTAATTAAIVPGSQLMPSKSPSTGTTEISSHESSHGTPSQTTAKNWELTASASHQPPGVYPQGHSDTTPILLTISLLSFFSVALLVILACVLWKKRIKPIVWPSLPDHKKTLEHLCKKPRKNLNVSFNPESFLDCQIHRVDDIQARDEVEGFLQDTFPQQLEESEKQRLGGDVQSPNCPSEDVVITPESFGRDSSLTCLAGNVSACDAPILSSSRSLDCRESGKNGPHVYQDLLLSLGTTNSTLPPPFSLQSGILTLNPVAQGQPILTSLGSNQEEAYVTMSSFYQNQ

SEQ ID NO: 18 - DNA, 1605 bp, Artificial Sequence
  source: /note="Description of Artificial Sequence: Synthetic Exemplary chimeric transmembrane sequence"
aactgggtgaatgtgatcagcgacctgaagaagatcgaggatctgatccagagcatgcacattgatgccaccctgtacacagaatctgatgtgcaccctagctgtaaagtgaccgccatgaagtgttttctgctggagctgcaggtgatttctctggaaagcggagatgcctctatccacgacacagtggagaatctgatcatcctggccaacaatagcctgagcagcaatggcaatgtgacagagtctggctgtaaggagtgtgaggagctggaggagaagaacatcaaggagtttctgcagagctttgtgcacatcgtgcagatgttcatcaatacaagcagcggtgggggctcaggcggaggaggctctggcggaggcggaagcgggggagggggctcaggcggcgggtccttgcagattacatgccctcctccaatgtctgtggagcacgccgatatttgggtgaagtcctacagcctgtacagcagagagagatacatctgcaacagcggctttaagagaaaggccggcacctcttctctgacagagtgcgtgctgaataaggccacaaatgtggcccactggacaacacctagcctgaagtgcattagagatcctgccctggtccaccagaggcctgcccctccatctacagtgacaacagccggagtgacacctcagcctgaatctctgagcccttctggaaaagaacctgccgccagctctcctagctctaataataccgccgccacaacagccgccattgtgcctggatctcagctgatgcctagcaagtctcctagcacaggcacaacagagatcagcagccacgaatcttctcacggaacaccttctcagaccaccgccaagaattgggagctgacagcctctgcctctcaccagcctccaggagtgtatcctcagggccactctgatacaacacccatcctgctgaccatcagcatcctgagcttcttcagcgtggccctgctggtgatcctggcctgcgtgctgtggaagaagaggatcaagcccatcgtgtggcccagcctgcccgaccacaagaagaccctggagcacctgtgtaagaagcccaggaagaacctgaacgtgagcttcaaccccgagagcttcctggactgccagatccacagggtggacgacatccaggccagggacgaggtggagggcttcctgcaggacaccttcccccagcagctggaggagagcgagaagcagaggctgggcggcgacgtgcagagccccaactgccccagcgaggacgtggtgatcacccccgagagcttcggcagggacagcagcctgacctgcctggccggcaacgtgagcgcctgcgacgcccccatcctgagcagcagcaggagcctggactgcagggagagcggcaagaacggcccccacgtgtaccaggacctgctgctgagcctgggcaccaccaacagcaccctgccaccccccttcagcctgcagagcggcatcctgaccctgaaccccgtggcccagggccagcccatcctgaccagcctgggcagcaaccaggaggaggcctacgtgaccatgagcagcttctaccagaaccag

SEQ ID NO: 19 - protein, 539 aa, Artificial Sequence
  source: /note="Description of Artificial Sequence: Synthetic Exemplary chimeric transmembrane protein sequence"
NWVNVISDLKKIEDLIQSMHIDATLYTESDVHPSCKVTAMKCFLLELQVISLESGDASIHDTVENLIILANNSLSSNGNVTESGCKECEELEEKNIKEFLQSFVHIVQMFINTSSGGGSGGGGSGGGGSGGGGSGGGSLQITCPPPMSVEHADIWVKSYSLYSRERYICNSGFKRKAGTSSLTECVLNKATNVAHWTTPSLKCIRDPALVHQRPAPPSTVTTAGVTPQPESLSPSGKEPAASSPSSNNTAATTAAIVPGSQLMPSKSPSTGTTEISSHESSHGTPSQTTAKNWELTASASHQPPGVYPQGHSDTTPILLPPCLTISILSFFSVALLVILACVLWKKRIKPIVWPSLPDHKKTLEHLCKKPRKNLNVSFNPESFLDCQIHRVDDIQARDEVEGFLQDTFPQQLEESEKQRLGGDVQSPNCPSEDVVITPESFGRDSSLTCLAGNVSACDAPILSSSRSLDCRESGKNGPHVYQDLLLSLGTTNSTLPPPFSLQSGILTLNPVAQGQPILTSLGSNQEEAYVTMSSFYQNQ

SEQ ID NO: 20 - DNA, 1617 bp, Artificial Sequence
  source: /note="Description of Artificial Sequence: Synthetic Exemplary chimeric transmembrane sequence"
aactgggtgaatgtgatcagcgacctgaagaagatcgaggatctgatccagagcatgcacattgatgccaccctgtacacagaatctgatgtgcaccctagctgtaaagtgaccgccatgaagtgttttctgctggagctgcaggtgatttctctggaaagcggagatgcctctatccacgacacagtggagaatctgatcatcctggccaacaatagcctgagcagcaatggcaatgtgacagagtctggctgtaaggagtgtgaggagctggaggagaagaacatcaaggagtttctgcagagctttgtgcacatcgtgcagatgttcatcaatacaagcagcggtgggggctcaggcggaggaggctctggcggaggcggaagcgggggagggggctcaggcggcgggtccttgcagattacatgccctcctccaatgtctgtggagcacgccgatatttgggtgaagtcctacagcctgtacagcagagagagatacatctgcaacagcggctttaagagaaaggccggcacctcttctctgacagagtgcgtgctgaataaggccacaaatgtggcccactggacaacacctagcctgaagtgcattagagatcctgccctggtccaccagaggcctgcccctccatctacagtgacaacagccggagtgacacctcagcctgaatctctgagcccttctggaaaagaacctgccgccagctctcctagctctaataataccgccgccacaacagccgccattgtgcctggatctcagctgatgcctagcaagtctcctagcacaggcacaacagagatcagcagccacgaatcttctcacggaacaccttctcagaccaccgccaagaattgggagctgacagcctctgcctctcaccagcctccaggagtgtatcctcagggccactctgatacaacacccatcctgctgccaccctgtttaaccatcagcatcctgagcttcttcagcgtggccctgctggtgatcctggcctgcgtgctgtggaagaagaggatcaagcccatcgtgtggcccagcctgcccgaccacaagaagaccctggagcacctgtgtaagaagcccaggaagaacctgaacgtgagcttcaaccccgagagcttcctggactgccagatccacagggtggacgacatccaggccagggacgaggtggagggcttcctgcaggacaccttcccccagcagctggaggagagcgagaagcagaggctgggcggcgacgtgcagagccccaactgccccagcgaggacgtggtgatcacccccgagagcttcggcagggacagcagcctgacctgcctggccggcaacgtgagcgcctgcgacgcccccatcctgagcagcagcaggagcctggactgcagggagagcggcaagaacggcccccacgtgtaccaggacctgctgctgagcctgggcaccaccaacagcaccctgccaccccccttcagcctgcagagcggcatcctgaccctgaaccccgtggcccagggccagcccatcctgaccagcctgggcagcaaccaggaggaggcctacgtgaccatgagcagcttctaccagaaccag

SEQ ID NO: 21 - protein, 18 aa, Homo sapiens
MDWTWILFLVAAATRVHS

SEQ ID NO: 22 - protein, 114 aa, Homo sapiens
NWVNVISDLKKIEDLIQSMHIDATLYTESDVHPSCKVTAMKCFLLELQVISLESGDASIHDTVENLIILANNSLSSNGNVTESGCKECEELEEKNIKEFLQSFVHIVQMFINTS

SEQ ID NO: 23 - DNA, 342 bp, Homo sapiens
aactgggtgaatgtaataagtgatttgaaaaaaattgaagatcttattcaatctatgcatattgatgctactttatatacggaaagtgatgttcaccccagttgcaaagtaacagcaatgaagtgctttctcttggagttacaagttatttcacttgagtccggagatgcaagtattcatgatacagtagaaaatctgatcatcctagcaaacaacagtttgtcttctaatgggaatgtaacagaatctggatgcaaagaatgtgaggaactggaggaaaaaaatattaaagaatttttgcagagttttgtacatattgtccaaatgttcatcaacacttct

SEQ ID NO: 24 - protein, 135 aa, Homo sapiens
MVLGTIDLCSCFSAGLPKTEANWVNVISDLKKIEDLIQSMHIDATLYTESDVHPSCKVTAMKCFLLELQVISLESGDASIHDTVENLIILANNSLSSNGNVTESGCKECEELEEKNIKEFLQSFVHIVQMFINTS

SEQ ID NO: 25 - DNA, 408 bp, Homo sapiens
atggtattgggaaccatagatttgtgcagctgtttcagtgcagggcttcctaaaacagaagccaactgggtgaatgtaataagtgatttgaaaaaaattgaagatcttattcaatctatgcatattgatgctactttatatacggaaagtgatgttcaccccagttgcaaagtaacagcaatgaagtgctttctcttggagttacaagttatttcacttgagtccggagatgcaagtattcatgatacagtagaaaatctgatcatcctagcaaacaacagtttgtcttctaatgggaatgtaacagaatctggatgcaaagaatgtgaggaactggaggaaaaaaatattaaagaatttttgcagagttttgtacatattgtccaaatgttcatcaacacttcttga

SEQ ID NO: 26 - protein, 114 aa, Mus musculus
NWIDVRYDLEKIESLIQSIHIDTTLYTDSDFHPSCKVTAMNCFLLELQVILHEYSNMTLNETVRNVLYLANSTLSSNKNVAESGCKECEELEEKTFTEFLQSFIRIVQMFINTS

SEQ ID NO: 27 - DNA, 342 bp, Mus musculus
aactggatagatgtaagatatgacctggagaaaattgaaagccttattcaatctattcatattgacaccactttatacactgacagtgactttcatcccagttgcaaagttactgcaatgaactgctttctcctggaattgcaggttattttacatgagtacagtaacatgactcttaatgaaacagtaagaaacgtgctctaccttgcaaacagcactctgtcttctaacaagaatgtagcagaatctggctgcaaggaatgtgaggagctggaggagaaaaccttcacagagtttttgcaaagctttatacgcattgtccaaatgttcatcaacacgtcc

SEQ ID NO: 28 - protein, 114 aa, Mus musculus; identical to SEQ ID NO: 26

SEQ ID NO: 29 - DNA, 342 bp, Mus musculus; identical to SEQ ID NO: 27

SEQ ID NO: 30 - protein, 439 aa, Homo sapiens
ESGYAQNGDLEDAELDDYSFSCYSQLEVNGSQHSLTCAFEDPDVNITNLEFEICGALVEVKCLNFRKLQEIYFIETKKFLLIGKSNICVKVGEKSLTCKKIDLTTIVKPEAPFDLSVVYREGANDFVVTFNTSHLQKKYVKVLMHDVAYRQEKDENKWTHVNLSSTKLTLLQRKLQPAAMYEIKVRSIPDHYFKGFWSEWSPSYYFRTPEINNSSGEMDPILLTISILSFFSVALLVILACVLWKKRIKPIVWPSLPDHKKTLEHLCKKPRKNLNVSFNPESFLDCQIHRVDDIQARDEVEGFLQDTFPQQLEESEKQRLGGDVQSPNCPSEDVVITPESFGRDSSLTCLAGNVSACDAPILSSSRSLDCRESGKNGPHVYQDLLLSLGTTNSTLPPPFSLQSGILTLNPVAQGQPILTSLGSNQEEAYVTMSSFYQNQ

SEQ ID NO: 31 - DNA, 1317 bp, Homo sapiens
gaaagtggctatgctcaaaatggagacttggaagatgcagaactggatgactactcattctcatgctatagccagttggaagtgaatggatcgcagcactcactgacctgtgcttttgaggacccagatgtcaacatcaccaatctggaatttgaaatatgtggggccctcgtggaggtaaagtgcctgaatttcaggaaactacaagagatatatttcatcgagacaaagaaattcttactgattggaaagagcaatatatgtgtgaaggttggagaaaagagtctaacctgcaaaaaaatagacctaaccactatagttaaacctgaggctccttttgacctgagtgtcgtctatcgggaaggagccaatgactttgtggtgacatttaatacatcacacttgcaaaagaagtatgtaaaagttttaatgcacgatgtagcttaccgccaggaaaaggatgaaaacaaatggacgcatgtgaatttatccagcacaaagctgacactcctgcagagaaagctccaaccggcagcaatgtatgagattaaagttcgatccatccctgatcactattttaaaggcttctggagtgaatggagtccaagttattacttcagaactccagagatcaataatagctcaggggagatggatcctatcttactaaccatcagcattttgagttttttctctgtcgctctgttggtcatcttggcctgtgtgttatggaaaaaaaggattaagcctatcgtatggcccagtctccccgatcataagaagactctggaacatctttgtaagaaaccaagaaaaaatttaaatgtgagtttcaatcctgaaagtttcctggactgccagattcatagggtggatgacattcaagctagagatgaagtggaaggttttctgcaagatacgtttcctcagcaactagaagaatctgagaagcagaggcttggaggggatgtgcagagccccaactgcccatctgaggatgtagtcatcactccagaaagctttggaagagattcatccctcacatgcctggctgggaatgtcagtgcatgtgacgcccctattctctcctcttccaggtccctagactgcagggagagtggcaagaatgggcctcatgtgtaccaggacctcctgcttagccttgggactacaaacagcacgctgccccctccattttctctccaatctggaatcctgacattgaacccagttgctcagggtcagcccattcttacttccctgggatcaaatcaagaagaagcatatgtcaccatgtccagcttctaccaaaaccag

SEQ ID NO: 32 - protein, 439 aa, Mus musculus
ESGNAQDGDLEDADADDHSFWCHSQLEVDGSQHLLTCAFNDSDINTANLEFQICGALLRVKCLTLNKLQDIYFIKTSEFLLIGSSNICVKLGQKNLTCKNMAINTIVKAEAPSDLKVVYRKEANDFLVTFNAPHLKKKYLKKVKHDVAYRPARGESNWTHVSLFHTRTTIPQRKLRPKAMYEIKVRSIPHNDYFKGFWSEWSPSSTFETPEPKNQGGWDPVLPSVTILSLFSVFLLVILAHVLWKKRIKPVVWPSLPDHKKTLEQLCKKPKTSLNVSFNPESFLDCQIHEVKGVEARDEVESFLPNDLPAQPEELETQGHRAAVHSANRSPETSVSPPETVRRESPLRCLARNLSTCNAPPLLSSRSPDYRDGDRNRPPVYQDLLPNSGNTNVPVPVPQPLPFQSGILIPVSQRQPISTSSVLNQEEAYVTMSSFYQNK

SEQ ID NO: 33 - DNA, 1317 bp, Mus musculus
gaaagtggaaatgcccaggatggagacctagaagatgcagacgcggacgatcactccttctggtgccacagccagttggaagtggatggaagtcaacatttattgacttgtgcttttaatgactcagacatcaacacagctaatctggaatttcaaatatgtggggctcttttacgagtgaaatgcctaactcttaacaagctgcaagatatatattttataaagacatcagaattcttactgattggtagcagcaatatatgtgtgaagcttggacaaaagaatttaacttgcaaaaatatggctataaacacaatagttaaagccgaggctccctctgacctgaaagtcgtttatcgcaaagaagcaaatgattttttggtgacatttaatgcacctcacttgaaaaagaaatatttaaaaaaagtaaagcatgatgtggcctaccgcccagcaaggggtgaaagcaactggacgcatgtatctttattccacacaagaacaacaatcccacagagaaaactacgaccaaaagcaatgtatgaaatcaaagtccgatccattccccataacgattacttcaaaggcttctggagcgagtggagtccaagttctaccttcgaaactccagaacccaagaatcaaggaggatgggatcctgtcttgccaagtgtcaccattctgagtttgttctctgtgtttttgttggtcatcttagcccatgtgctatggaaaaaaaggattaaacctgtcgtatggcctagtctccccgatcataagaaaactctggaacaactatgtaagaagccaaaaacgagtctgaatgtgagtttcaatcccgaaagtttcctggactgccagattcatgaggtgaaaggcgttgaagccagggacgaggtggaaagttttctgcccaatgatcttcctgcacagccagaggagttggagacacagggacacagagccgctgtacacagtgcaaaccgctcgcctgagacttcagtcagcccaccagaaacagttagaagagagtcacccttaagatgcctggctagaaatctgagtacctgcaatgcccctccactcctttcctctaggtcccctgactacagagatggtgacagaaataggcctcctgtgtatcaagacttgctgccaaactctggaaacacaaatgtccctgtccctgtccctcaaccattgcctttccagtcgggaatcctgataccagtttctcagagacagcccatctccacttcctcagtactgaatcaagaagaagcgtatgtcaccatgtctagtttttaccaaaacaaa

SEQ ID NO: 34 - protein, 266 aa, Mus musculus
ESGNAQDGDLEDADADDHSFWCHSQLEVDGSQHLLTCAFNDSDINTANLEFQICGALLRVKCLTLNKLQDIYFIKTSEFLLIGSSNICVKLGQKNLTCKNMAINTIVKAEAPSDLKVVYRKEANDFLVTFNAPHLKKKYLKKVKHDVAYRPARGESNWTHVSLFHTRTTIPQRKLRPKAMYEIKVRSIPHNDYFKGFWSEWSPSSTFETPEPKNQGGWDPVLPSVTILSLFSVFLLVILAHVLWKKRIKPVVWPSLPDHKKTLEQL

SEQ ID NO: 35 - DNA, 861 bp, Mus musculus
atgatggctctgggtagagctttcgctatagttttctgcttaattcaagctgtttctggagaaagtggaaatgcccaggatggagacctagaagatgcagacgcggacgatcactccttctggtgccacagccagttggaagtggatggaagtcaacatttattgacttgtgcttttaatgactcagacatcaacacagctaatctggaatttcaaatatgtggggctcttttacgagtgaaatgcctaactcttaacaagctgcaagatatatattttataaagacatcagaattcttactgattggtagcagcaatatatgtgtgaagcttggacaaaagaatttaacttgcaaaaatatggctataaacacaatagttaaagccgaggctccctctgacctgaaagtcgtttatcgcaaagaagcaaatgattttttggtgacatttaatgcacctcacttgaaaaagaaatatttaaaaaaagtaaagcatgatgtggcctaccgcccagcaaggggtgaaagcaactggacgcatgtatctttattccacacaagaacaacaatcccacagagaaaactacgaccaaaagcaatgtatgaaatcaaagtccgatccattccccataacgattacttcaaaggcttctggagcgagtggagtccaagttctaccttcgaaactccagaacccaagaatcaaggaggatgggatcctgtcttgccaagtgtcaccattctgagtttgttctctgtgtttttgttggtcatcttagcccatgtgctatggaaaaaaaggattaaacctgtcgtatggcctagtctccccgatcataagaaaactctggaacaactatag

SEQ ID NO: 36 - protein, 62 aa, Homo sapiens
CPPPMSVEHADIWVKSYSLYSRERYICNSGFKRKAGTSSLTECVLNKATNVAHWTTPSLKCI

SEQ ID NO: 37 - protein, 62 aa, Homo sapiens; identical to SEQ ID NO: 36

SEQ ID NO: 38 - protein, 62 aa, Mus musculus
CPPPVSIEHADIRVKNYSVNSRERYVCNSGFKRKAGTSTLIECVINKNTNVAHWTTPSLKCI

SEQ ID NO: 39 - protein, 62 aa, Mus musculus; identical to SEQ ID NO: 38

SEQ ID NO: 40 - protein, 59 aa, Gallus gallus
CPRLSTTEFADVAAETYPLKTKLRYECDSGYRRRSGNTLTIRCQNVSGTASWVHDELVC

SEQ ID NO: 41 - protein, 175 aa, Homo sapiens
ITCPPPMSVEHADIWVKSYSLYSRERYICNSGFKRKAGTSSLTECVLNKATNVAHWTTPSLKCIRDPALVHQRPAPPSTVTTAGVTPQPESLSPSGKEPAASSPSSNNTAATTAAIVPGSQLMPSKSPSTGTTEISSHESSHGTPSQTTAKNWELTASASHQPPGVYPQGHSDTT

SEQ ID NO: 42 - protein, 25 aa, Mus musculus
PVLPSVTILSLFSVFLLVILAHVLW

SEQ ID NO: 43 - skipped

SEQ ID NO: 44 - protein, 25 aa, Macaca fascicularis
PILLTISLLSFFSVALLVILACVLW

SEQ ID NO: 45 - protein, 195 aa, Homo sapiens
KKRIKPIVWPSLPDHKKTLEHLCKKPRKNLNVSFNPESFLDCQIHRVDDIQARDEVEGFLQDTFPQQLEESEKQRLGGDVQSPNCPSEDVVITPESFGRDSSLTCLAGNVSACDAPILSSSRSLDCRESGKNGPHVYQDLLLSLGTTNSTLPPPFSLQSGILTLNPVAQGQPILTSLGSNQEEAYVTMSSFYQNQ

SEQ ID NO: 46 - protein, 195 aa, Mus musculus
KKRIKPVVWPSLPDHKKTLEQLCKKPKTSLNVSFNPESFLDCQIHEVKGVEARDEVESFLPNDLPAQPEELETQGHRAAVHSANRSPETSVSPPETVRRESPLRCLARNLSTCNAPPLLSSRSPDYRDGDRNRPPVYQDLLPNSGNTNVPVPVPQPLPFQSGILIPVSQRQPISTSSVLNQEEAYVTMSSFYQNK

SEQ ID NO: 47 - protein, 4 aa, Artificial Sequence
  source: /note="Description of Artificial Sequence: Synthetic Linker sequence"
SGGS

SEQ ID NO: 48 - protein, 5 aa, Artificial Sequence
  source: /note="Description of Artificial Sequence: Synthetic Linker sequence"
SGGGS

SEQ ID NO: 49 - protein, 6 aa, Artificial Sequence
  source: /note="Description of Artificial Sequence: Synthetic Linker sequence"
SGGGGS

SEQ ID NO: 50 - protein, 15 aa, Artificial Sequence
  source: /note="Description of Artificial Sequence: Synthetic Linker sequence"
SGGGGSGGGGSGGGG

SEQ ID NO: 51 - protein, 19 aa, Artificial Sequence
  source: /note="Description of Artificial Sequence: Synthetic Linker sequence"
ASTKGPSVFPLAPSSSGSG

SEQ ID NO: 52 - protein, 15 aa, Artificial Sequence
  source: /note="Description of Artificial Sequence: Synthetic Linker sequence"
GGGGSGGGGSGGGGS

SEQ ID NO: 53 - protein, 23 aa, Artificial Sequence
  source: /note="Description of Artificial Sequence: Synthetic Linker sequence"
GGGSGGGGSGGGGSGGGGSGGGS

SEQ ID NO: 54 - protein, 18 aa, Artificial Sequence
  source: /note="Description of Artificial Sequence: Synthetic Linker sequence"
GSTSGSGKPGSGEGSTKG

SEQ ID NO: 55 - DNA, 54 bp, Artificial Sequence
  source: /note="Description of Artificial Sequence: Synthetic Linker sequence"
ggcagcaccagcggcagcggcaaaccgggcagcggcgaaggcagcaccaaaggc

SEQ ID NO: 56 - protein, 25 aa, Artificial Sequence
  source: /note="Description of Artificial Sequence: Synthetic Linker sequence"
GGGGSGGGGSGGGGSGGGGSGGGGS

SEQ ID NO: 57 - DNA, 75 bp, Artificial Sequence
  source: /note="Description of Artificial Sequence: Synthetic Linker sequence"
ggcggtggtggttctggaggcggtggcagcggtggaggtggctcaggaggaggaggtagcggcggcggagggagt

SEQ ID NO: 58 - protein, 233 aa, Homo sapiens
AEPKSPDKTHTCPPCPAPPVAGPSVFLFPPKPKDTLMIARTPEVTCWVDVSHEDPEVKFNWYVDGVEVHNAKTKPREEQYNSTYRVVSVLTVLHQDWLNGKEYKCKVSNKALPAPIEKTISKAKGQPREPQVYTLPPSRDELTKNQVSLTCLVKGFYPSDIAVEWESNGQPENNYKTTPPVLDSDGSFFLYSKLTVDKSRWQQGNVFSCSVMHEALHNHYTQKSLSLSPGKKD

SEQ ID NO: 59 - protein, 46 aa, Homo sapiens
TTTPAPRPPTPAPTIASQPLSLRPEACRPAAGGAVHTRGLDFACDI

SEQ ID NO: 60 - protein, 20 aa, Homo sapiens
AEPKSPDKTHTCPPCPKDPK

SEQ ID NO: 61 - protein, 220 aa, Homo sapiens
MLRLLLALNLFPSIQVTGNKILVKQSPMLVAYDNAVNLSCKYSYNLFSREFRASLHKGLDSAVEVCVVYGNYSQQLQVYSKTGFNCDGKLGNESVTFYLQNLYVNQTDIYFCKIEVMYPPPYLDNEKSNGTIIHVKGKHLCPSPLFPGPSKPFWVLVVVGGVLACYSLLVTVAFIIFWVRSKRSRLLHSDYMNMTPRRPGPTRKHYQPYAPPRDFAAYRS

SEQ ID NO: 62 - protein, 164 aa, Homo sapiens
MKWKALFTAAILQAQLPITEAQSFGLLDPKLCYLLDGILFIYGVILTALFLRVKFSRSADAPAYQQGQNQLYNELNLGRREEYDVLDKRRGRDPEMGGKPQRRKNPQEGLYNELQKDKMAEAYSEIGMKGERRRGKGHDGLYQGLSTATKDTYDALHMQALPPR

SEQ ID NO: 63 - protein, 23 aa, Homo sapiens
LGLLVAGVLVLLVSLGVAIHLCC

SEQ ID NO: 64 - protein, 26 aa, Homo sapiens
VAAILGLGLVLGLLGPLAILLALYLL

SEQ ID NO: 65 - protein, 25 aa, Homo sapiens
ALIVLGGVAGLLLFIGLGIFFCVRC

SEQ ID NO: 66 - protein, 23 aa, Homo sapiens
LCYLLDGILFIYGVILTALFLRV

SEQ ID NO: 67 - protein, 26 aa, Homo sapiens
WVLVVVGGVLACYSLLVTVAFIIFWV

SEQ ID NO: 68 - protein, 24 aa, Homo sapiens
IYIWAPLAGTCGVLLLSLVITLYC

SEQ ID NO: 69 - protein, 24 aa, Homo sapiens
ALPAALAVISFLLGLGLGVACVLA

SEQ ID NO: 70 - protein, 220 aa, Homo sapiens; identical to SEQ ID NO: 61

SEQ ID NO: 71 - protein, 255 aa, Homo sapiens
MGNSCYNIVATLLLVLNFERTRSLQDPCSNCPAGTFCDNNRNQICSPCPPNSFSSAGGQRTCDICRQCKGVFRTRKECSSTSNAECDCTPGFHCLGAGCSMCEQDCKQGQELTKKGCKDCCFGTFNDQKRGICRPWTNCSLDGKSVLVNGTKERDVVCGPSPADLSPGASSVTPPAPAREPGHSPQIISFFLALTSTALLFLLFFLTLRFSVVKRGRKKLLYIFKQPFMRPVQTTQEEDGCSCRFPEEEEGGCEL

SEQ ID NO: 72 - protein, 164 aa, Homo sapiens; identical to SEQ ID NO: 62

SEQ ID NO: 73 - protein, 113 aa, Homo sapiens
LRVKFSRSADAPAYQQGQNQLYNELNLGRREEYDVLDKRRGRDPEMGGKPRRKNPQEGLYNELQKDKMAEAYSEIGMKGERRRGKGHDGLYQGLSTATKDTYDALHMQALPPR

SEQ ID NO: 74 - DNA, 339 bp, Homo sapiens
ctgagagtgaagttcagcaggagcgcagacgcccccgcgtaccagcagggccagaaccagctctataacgagctcaatctaggacgaagagaggagtacgatgttttggacaagagacgtggccgggaccctgagatggggggaaagccgagaaggaagaaccctcaggaaggcctgtacaatgaactgcagaaagataagatggcggaggcctacagtgagattgggatgaaaggcgagcgccggaggggcaaggggcacgatggcctttaccagggtctcagtacagccaccaaggacacctacgacgcccttcacatgcaggccctgccccctcgc

SEQ ID NO: 75 - protein, 233 aa, Homo sapiens; identical to SEQ ID NO: 58

SEQ ID NO: 76 - protein, 46 aa, Homo sapiens; identical to SEQ ID NO: 59

SEQ ID NO: 77 - protein, 20 aa, Homo sapiens
AEPKSPDKTHTCPPCPKDPK

SEQ ID NO: 78 - DNA, 17 bp, Homo sapiens
aaataaaatacgaaatg

SEQ ID NO: 79 - protein, 28 aa, Artificial Sequence
  source: /note="Description of Artificial Sequence: Synthetic IL7RA MCP insert sequence"
PILLTMCPISILSFFSVALLVILACVLW

SEQ ID NO: 80 - DNA, 84 bp, Artificial Sequence
  source: /note="Description of Artificial Sequence: Synthetic IL7RA MCP insert sequence"
cccatcctgctgaccatgtgccccatcagcatcctgagcttcttcagcgtggccctgctggtgatcctggcctgcgtgctgtgg

SEQ ID NO: 81 - DNA, 66 bp, Homo sapiens
atgctcctgctcgtgacttcacttcttctctgtgaactcccacaccccgcgtttttgcttatccct

SEQ ID NO: 82 - DNA, 586 bp, Homo sapiens
aagaagaggatcaagcccatcgtgtggcccagcctgcccgaccacaagaagaccctggagcacctgtgtaagaagcccaggaagaacctgaacgtgagcttcaaccccgagagcttcctggactgccagatccacagggtggacgacatccaggccagggacgaggtggagggcttcctgcaggacaccttcccccagcagctggaggagagcgagaagcagaggctgggcggcgacgtgcagagccccaactgccccagcgaggacgtggtgatcacccccgagagcttcggcagggacagcagcctgacctgcctggccggcaacgtgagcgcctgcgacgcccccatcctgagcagcagcaggagcctggactgcagggagagcggcaagaacggcccccacgtgtaccaggacctgctgctgagcctgggcaccaccaacagcaccctgccaccccccttcagcctgcagagcggcatcctgaccctgaaccccgtggcccagggccagcccatcctgaccagcctgggcagcaaccaggaggaggcctacgtgaccatgagcagcttctaccagaaccags

SEQ ID NO: 83 - protein, 538 aa, Artificial Sequence
  source: /note="Description of Artificial Sequence: Synthetic Exemplary chimeric transmembrane protein sequence"
NWVNVISDLKKIEDLIQSMHIDATLYTESDVHPSCKVTAMKCFLLELQVISLESGDASIHDTVENLIILANNSLSSNGNVTESGCKECEELEEKNIKEFLQSFVHIVQMFINTSSGGGSGGGGSGGGGSGGGGSGGGSLQITCPPPMSVEHADIWVKSYSLYSRERYICNSGFKRKAGTSSLTECVLNKATNVAHWTTPSLKCIRDPALVHQRPAPPSTVTTAGVTPQPESLSPSGKEPAASSPSSNNTAATTAAIVPGSQLMPSKSPSTGTTEISSHESSHGTPSQTTAKNWELTASASHQPPGVYPQGHSDTTPILLTCPTISILSFFSVALLVILACVLWKKRIKPIVWPSLPDHKKTLEHLCKKPRKNLNVSFNPESFLDCQIHRVDDIQARDEVEGFLQDTFPQQLEESEKQRLGGDVQSPNCPSEDVVITPESFGRDSSLTCLAGNVSACDAPILSSSRSLDCRESGKNGPHVYQDLLLSLGTTNSTLPPPFSLQSGILTLNPVAQGQPILTSLGSNQEEAYVTMSSFYQNQ

SEQ ID NO: 84 - DNA, 1614 bp, Artificial Sequence
  source: /note="Description of Artificial Sequence: Synthetic Exemplary chimeric transmembrane sequence"
aactgggtgaatgtgatcagcgacctgaagaagatcgaggatctgatccagagcatgcacattgatgccaccctgtacacagaatctgatgtgcaccctagctgtaaagtgaccgccatgaagtgttttctgctggagctgcaggtgatttctctggaaagcggagatgcctctatccacgacacagtggagaatctgatcatcctggccaacaatagcctgagcagcaatggcaatgtgacagagtctggctgtaaggagtgtgaggagctggaggagaagaacatcaaggagtttctgcagagctttgtgcacatcgtgcagatgttcatcaatacaagcagcggtgggggctcaggcggaggaggctctggcggaggcggaagcgggggagggggctcaggcggcgggtccttgcagattacatgccctcctccaatgtctgtggagcacgccgatatttgggtgaagtcctacagcctgtacagcagagagagatacatctgcaacagcggctttaagagaaaggccggcacctcttctctgacagagtgcgtgctgaataaggccacaaatgtggcccactggacaacacctagcctgaagtgcattagagatcctgccctggtccaccagaggcctgcccctccatctacagtgacaacagccggagtgacacctcagcctgaatctctgagcccttctggaaaagaacctgccgccagctctcctagctctaataataccgccgccacaacagccgccattgtgcctggatctcagctgatgcctagcaagtctcctagcacaggcacaacagagatcagcagccacgaatcttctcacggaacaccttctcagaccaccgccaagaattgggagctgacagcctctgcctctcaccagcctccaggagtgtatcctcagggccactctgatacaacacccatcctgctgacctgccccaccatcagcatcctgagcttcttcagcgtggccctgctggtgatcctggcctgcgtgctgtggaagaagaggatcaagcccatcgtgtggcccagcctgcccgaccacaagaagaccctggagcacctgtgtaagaagcccaggaagaacctgaacgtgagcttcaaccccgagagcttcctggactgccagatccacagggtggacgacatccaggccagggacgaggtggagggcttcctgcaggacaccttcccccagcagctggaggagagcgagaagcagaggctgggcggcgacgtgcagagccccaactgccccagcgaggacgtggtgatcacccccgagagcttcggcagggacagcagcctgacctgcctggccggcaacgtgagcgcctgcgacgcccccatcctgagcagcagcaggagcctggactgcagggagagcggcaagaacggcccccacgtgtaccaggacctgctgctgagcctgggcaccaccaacagcaccctgccaccccccttcagcctgcagagcggcatcctgaccctgaaccccgtggcccagggccagcccatcctgaccagcctgggcagcaaccaggaggaggcctacgtgaccatgagcagcttctaccagaaccag

SEQ ID NO: 85 - protein, 538 aa, Artificial Sequence
  source: /note="Description of Artificial Sequence: Synthetic Exemplary chimeric transmembrane protein sequence"
NWVNVISDLKKIEDLIQSMHIDATLYTESDVHPSCKVTAMKCFLLELQVISLESGDASIHDTVENLIILANNSLSSNGNVTESGCKECEELEEKNIKEFLQSFVHIVQMFINTSSGGGSGGGGSGGGGSGGGGSGGGSLQITCPPPMSVEHADIWVKSYSLYSRERYICNSGFKRKAGTSSLTECVLNKATNVAHWTTPSLKCIRDPALVHQRPAPPSTVTTAGVTPQPESLSPSGKEPAASSPSSNNTAATTAAIVPGSQLMPSKSPSTGTTEISSHESSHGTPSQTTAKNWELTASASHQPPGVYPQGHSDTTPILLMCPTISILSFFSVALLVILACVLWKKRIKPIVWPSLPDHKKTLEHLCKKPRKNLNVSFNPESFLDCQIHRVDDIQARDEVEGFLQDTFPQQLEESEKQRLGGDVQSPNCPSEDVVITPESFGRDSSLTCLAGNVSACDAPILSSSRSLDCRESGKNGPHVYQDLLLSLGTTNSTLPPPFSLQSGILTLNPVAQGQPILTSLGSNQEEAYVTMSSFYQNQ

SEQ ID NO: 86 - DNA, 1614 bp, Artificial Sequence
  source: /note="Description of Artificial Sequence: Synthetic Exemplary chimeric transmembrane sequence"
aactgggtgaatgtgatcagcgacctgaagaagatcgaggatctgatccagagcatgcacattgatgccaccctgtacacagaatctgatgtgcaccctagctgtaaagtgaccgccatgaagtgttttctgctggagctgcaggtgatttctctggaaagcggagatgcctctatccacgacacagtggagaatctgatcatcctggccaacaatagcctgagcagcaatggcaatgtgacagagtctggctgtaaggagtgtgaggagctggaggagaagaacatcaaggagtttctgcagagctttgtgcacatcgtgcagatgttcatcaatacaagcagcggtgggggctcaggcggaggaggctctggcggaggcggaagcgggggagggggctcaggcggcgggtccttgcagattacatgccctcctccaatgtctgtggagcacgccgatatttgggtgaagtcctacagcctgtacagcagagagagatacatctgcaacagcggctttaagagaaaggccggcacctcttctctgacagagtgcgtgctgaataaggccacaaatgtggcccactggacaacacctagcctgaagtgcattagagatcctgccctggtccaccagaggcctgcccctccatctacagtgacaacagccggagtgacacctcagcctgaatctctgagcccttctggaaaagaacctgccgccagctctcctagctctaataataccgccgccacaacagccgccattgtgcctggatctcagctgatgcctagcaagtctcctagcacaggcacaacagagatcagcagccacgaatcttctcacggaacaccttctcagaccaccgccaagaattgggagctgacagcctctgcctctcaccagcctccaggagtgtatcctcagggccactctgatacaacacccatcctgctgatgtgccccaccatcagcatcctgagcttcttcagcgtggccctgctggtgatcctggcctgcgtgctgtggaagaagaggatcaagcccatcgtgtggcccagcctgcccgaccacaagaagaccctggagcacctgtgtaagaagcccaggaagaacctgaacgtgagcttcaaccccgagagcttcctggactgccagatccacagggtggacgacatccaggccagggacgaggtggagggcttcctgcaggacaccttcccccagcagctggaggagagcgagaagcagaggctgggcggcgacgtgcagagccccaactgccccagcgaggacgtggtgatcacccccgagagcttcggcagggacagcagcctgacctgcctggccggcaacgtgagcgcctgcgacgcccccatcctgagcagcagcaggagcctggactgcagggagagcggcaagaacggcccccacgtgtaccaggacctgctgctgagcctgggcaccaccaacagcaccctgccaccccccttcagcctgcagagcggcatcctgaccctgaaccccgtggcccagggccagcccatcctgaccagcctgggcagcaaccaggaggaggcctacgtgaccatgagcagcttctaccagaaccag

SEQ ID NO: 87 - protein, 535 aa, Artificial Sequence
  source: /note="Description of Artificial Sequence: Synthetic Exemplary chimeric transmembrane protein sequence"
NWVNVISDLKKIEDLIQSMHIDATLYTESDVHPSCKVTAMKCFLLELQVISLESGDASIHDTVENLIILANNSLSSNGNVTESGCKECEELEEKNIKEFLQSFVHIVQMFINTSSGGGSGGGGSGGGGSGGGGSGGGSLQITCPPPMSVEHADIWVKSYSLYSRERYICNSGFKRKAGTSSLTECVLNKATNVAHWTTPSLKCIRDPALVHQRPAPPSTVTTAGVTPQPESLSPSGKEPAASSPSSNNTAATTAAIVPGSQLMPSKSPSTGTTEISSHESSHGTPSQTTAKNWELTASASHQPPGVYPQGHSDTTPILLTISILSFFSVEKAVILACVLWKKRIKPIVWPSLPDHKKTLEHLCKKPRKNLNVSFNPESFLDCQIHRVDDIQARDEVEGFLQDTFPQQLEESEKQRLGGDVQSPNCPSEDVVITPESFGRDSSLTCLAGNVSACDAPILSSSRSLDCRESGKNGPHVYQDLLLSLGTTNSTLPPPFSLQSGILTLNPVAQGQPILTSLGSNQEEAYVTMSSFYQNQ

SEQ ID NO: 88 - DNA, 1605 bp, Artificial Sequence
  source: /note="Description of Artificial Sequence: Synthetic Exemplary chimeric transmembrane sequence"
aactgggtgaatgtgatcagcgacctgaagaagatcgaggatctgatccagagcatgcacattgatgccaccctgtacacagaatctgatgtgcaccctagctgtaaagtgaccgccatgaagtgttttctgctggagctgcaggtgatttctctggaaagcggagatgcctctatccacgacacagtggagaatctgatcatcctggccaacaatagcctgagcagcaatggcaatgtgacagagtctggctgtaaggagtgtgaggagctggaggagaagaacatcaaggagtttctgcagagctttgtgcacatcgtgcagatgttcatcaatacaagcagcggtgggggctcaggcggaggaggctctggcggaggcggaagcgggggagggggctcaggcggcgggtccttgcagattacatgccctcctccaatgtctgtggagcacgccgatatttgggtgaagtcctacagcctgtacagcagagagagatacatctgcaacagcggctttaagagaaaggccggcacctcttctctgacagagtgcgtgctgaataaggccacaaatgtggcccactggacaacacctagcctgaagtgcattagagatcctgccctggtccaccagaggcctgcccctccatctacagtgacaacagccggagtgacacctcagcctgaatctctgagcccttctggaaaagaacctgccgccagctctcctagctctaataataccgccgccacaacagccgccattgtgcctggatctcagctgatgcctagcaagtctcctagcacaggcacaacagagatcagcagccacgaatcttctcacggaacaccttctcagaccaccgccaagaattgggagctgacagcctctgcctctcaccagcctccaggagtgtatcctcagggccactctgatacaacacccatcctgctgaccatcagcatcctgagcttcttcagcgtggagaaggccgtgatcctggcctgcgtgctgtggaagaagaggatcaagcccatcgtgtggcccagcctgcccgaccacaagaagaccctggagcacctgtgtaagaagcccaggaagaacctgaacgtgagcttcaaccccgagagcttcctggactgccagatccacagggtggacgacatccaggccagggacgaggtggagggcttcctgcaggacaccttcccccagcagctggaggagagcgagaagcagaggctgggcggcgacgtgcagagccccaactgccccagcgaggacgtggtgatcacccccgagagcttcggcagggacagcagcctgacctgcctggccggcaacgtgagcgcctgcgacgcccccatcctgagcagcagcaggagcctggactgcagggagagcggcaagaacggcccccacgtgtaccaggacctgctgctgagcctgggcaccaccaacagcaccctgccaccccccttcagcctgcagagcggcatcctgaccctgaaccccgtggcccagggccagcccatcctgaccagcctgggcagcaaccaggaggaggcctacgtgaccatgagcagcttctaccagaaccag

SEQ ID NO: 89 - protein, 535 aa, Artificial Sequence
  source: /note="Description of Artificial Sequence: Synthetic Exemplary chimeric transmembrane protein sequence"
NWVNVISDLKKIEDLIQSMHIDATLYTESDVHPSCKVTAMKCFLLELQVISLESGDASIHDTVENLIILANNSLSSNGNVTESGCKECEELEEKNIKEFLQSFVHIVQMFINTSSGGGSGGGGSGGGGSGGGGSGGGSLQITCPPPMSVEHADIWVKSYSLYSRERYICNSGFKRKAGTSSLTECVLNKATNVAHWTTPSLKCIRDPALVHQRPAPPSTVTTAGVTPQPESLSPSGKEPAASSPSSNNTAATTAAIVPGSQLMPSKSPSTGTTEISSHESSHGTPSQTTAKNWELTASASHQPPGVYPQGHSDTTPILLTISILSFFSVEKVVILACVLWKKRIKPIVWPSLPDHKKTLEHLCKKPRKNLNVSFNPESFLDCQIHRVDDIQARDEVEGFLQDTFPQQLEESEKQRLGGDVQSPNCPSEDVVITPESFGRDSSLTCLAGNVSACDAPILSSSRSLDCRESGKNGPHVYQDLLLSLGTTNSTLPPPFSLQSGILTLNPVAQGQPILTSLGSNQEEAYVTMSSFYQNQ

SEQ ID NO: 90 - DNA, 1605 bp, Artificial Sequence
  source: /note="Description of Artificial Sequence: Synthetic Exemplary chimeric transmembrane sequence"
aactgggtgaatgtgatcagcgacctgaagaagatcgaggatctgatccagagcatgcacattgatgccaccctgtacacagaatctgatgtgcaccctagctgtaaagtgaccgccatgaagtgttttctgctggagctgcaggtgatttctctggaaagcggagatgcctctatccacgacacagtggagaatctgatcatcctggccaacaatagcctgagcagcaatggcaatgtgacagagtctggctgtaaggagtgtgaggagctggaggagaagaacatcaaggagtttctgcagagctttgtgcacatcgtgcagatgttcatcaatacaagcagcggtgggggctcaggcggaggaggctctggcggaggcggaagcgggggagggggctcaggcggcgggtccttgcagattacatgccctcctccaatgtctgtggagcacgccgatatttgggtgaagtcctacagcctgtacagcagagagagatacatctgcaacagcggctttaagagaaaggccggcacctcttctctgacagagtgcgtgctgaataaggccacaaatgtggcccactggacaacacctagcctgaagtgcattagagatcctgccctggtccaccagaggcctgcccctccatctacagtgacaacagccggagtgacacctcagcctgaatctctgagcccttctggaaaagaacctgccgccagctctcctagctctaataataccgccgccacaacagccgccattgtgcctggatctcagctgatgcctagcaagtctcctagcacaggcacaacagagatcagcagccacgaatcttctcacggaacaccttctcagaccaccgccaagaattgggagctgacagcctctgcctctcaccagcctccaggagtgtatcctcagggccactctgatacaacacccatcctgctgaccatcagcatcctgagcttcttcagcgtggagaaggtggtgatcctggcctgcgtgctgtggaagaagaggatcaagcccatcgtgtggcccagcctgcccgaccacaagaagaccctggagcacctgtgtaagaagcccaggaagaacctgaacgtgagcttcaaccccgagagcttcctggactgccagatccacagggtggacgacatccaggccagggacgaggtggagggcttcctgcaggacaccttcccccagcagctggaggagagcgagaagcagaggctgggcggcgacgtgcagagccccaactgccccagcgaggacgtggtgatcacccccgagagcttcggcagggacagcagcctgacctgcctggccggcaacgtgagcgcctgcgacgcccccatcctgagcagcagcaggagcctggactgcagggagagcggcaagaacggcccccacgtgtaccaggacctgctgctgagcctgggcaccaccaacagcaccctgccaccccccttcagcctgcagagcggcatcctgaccctgaaccccgtggcccagggccagcccatcctgaccagcctgggcagcaaccaggaggaggcctacgtgaccatgagcagcttctaccagaaccag

SEQ ID NO: 91 - DNA, 54 bp, Homo sapiens
atggattggacctggattctgtttctggtggccgctgccacaagagtgcacagc

SEQ ID NO: 92 - protein, 26 aa, Artificial Sequence
  source: /note="Description of Artificial Sequence: Synthetic Linker sequence"
SGGGSGGGGSGGGGSGGGGSGGGSLQ

SEQ ID NO: 93 - protein, 22 aa, Homo sapiens
MLLLVTSLLLCELPHPAFLLIP

SEQ ID NO: 94 - DNA, 66 bp, Homo sapiens
atgcttctcctggtgacaagccttctgctctgtgagttaccacacccagcattcctcctgattcct

SEQ ID NO: 95 - protein, 242 aa, Artificial Sequence
  source: /note="Description of Artificial Sequence: Synthetic Anti-CD19 scFv sequence"
DIQMTQTTSSLSASLGDRVTISCRASQDISKYLNWYQQKPDGTVKLLIYHTSRLHSGVPSRFSGSGSGTDYSLTISNLEQEDIATYFCQQGNTLPYTFGGGTKLEITGGGGSGGGGSGGGGSEVKLQESGPGLVAPSQSLSVTCTVSGVSLPDYGVSWIRQPPRKGLEWLGVIWGSETTYYNSALKSRLTIIKDNSKSQVFLKMNSLQTDDTAIYYCAKHYYYGGSYAMDYWGQGTSVTVSS

SEQ ID NO: 96 - DNA, 726 bp, Artificial Sequence
  source: /note="Description of Artificial Sequence: Synthetic Anti-CD19 scFv sequence"
gacatccagatgacccagaccaccagcagcctgagcgccagcctgggcgatagagtgaccatcagctgcagagccagccaggacatcagcaagtacctgaactggtatcagcagaaacccgacggcaccgtgaagctgctgatctaccacaccagcagactgcacagcggcgtgcccagcagattttctggcagcggctccggcaccgactacagcctgaccatctccaacctggaacaggaagatatcgctacctacttctgtcagcaaggcaacaccctgccctacaccttcggcggaggcaccaagctggaaatcacaggcggcggaggatctggcggaggcggaagtggcggagggggatctgaagtgaaactgcaggaaagcggccctggcctggtggccccatctcagtctctgagcgtgacctgtaccgtgtccggcgtgtccctgcctgactatggcgtgtcctggatcagacagccccccagaaagggcctggaatggctgggagtgatctggggcagcgagacaacctactacaacagcgccctgaagtcccggctgaccatcatcaaggacaactccaagagccaggtgttcctgaagatgaacagcctgcagaccgacgacaccgccatctactactgcgccaagcactactactacggcggcagctacgccatggactactggggccagggcacaagcgtgaccgtgtctagc

SEQ ID NO: 97 - protein, 57 aa, Homo sapiens
LDNEKSNGTIIHVKGKHLCPSPLFPGPSKPFWVLVVVGGVLACYSLLVTVAFIIFWV

SEQ ID NO: 98 - DNA, 171 bp, Homo sapiens
ctagacaatgagaagagcaatggaaccattatccatgtgaaagggaaacacctttgtccaagtcccctatttcccggaccttctaagcccttttgggtgctggtggtggttggtggagtcctggcttgctatagcttgctagtaacagtggcctttattattttctgggtg

SEQ ID NO: 99 - DNA, 123 bp, Homo sapiens
aggagtaagaggagcaggctcctgcacagtgactacatgaacatgactccccgccgccccgggcccacccgcaagcattaccagccctatgccccaccacgcgacttcgcagcctatcgctcc

SEQ ID NO: 100 - DNA, 1396 bp, Artificial Sequence
  source: /note="Description of Artificial Sequence: Synthetic CD19 CAR DNA sequence"
gaacagaagctgataagtgaggaggacttggacatccagatgacccagaccaccagcagcctgagcgccagcctgggcgatagagtgaccatcagctgcagagccagccaggacatcagcaagtacctgaactggtatcagcagaaacccgacggcaccgtgaagctgctgatctaccacaccagcagactgcacagcggcgtgcccagcagattttctggcagcggctccggcaccgactacagcctgaccatctccaacctggaacaggaagatatcgctacctacttctgtcagcaaggcaacaccctgccctacaccttcggcggaggcaccaagctggaaatcacaggcggcggaggatctggcggaggcggaagtggcggagggggatctgaagtgaaactgcaggaaagcggccctggcctggtggccccatctcagtctctgagcgtgacctgtaccgtgtccggcgtgtccctgcctgactatggcgtgtcctggatcagacagccccccagaaagggcctggaatggctgggagtgatctggggcagcgagacaacctactacaacagcgccctgaagtcccggctgaccatcatcaaggacaactccaagagccaggtgttcctgaagatgaacagcctgcagaccgacgacaccgccatctactactgcgccaagcactactactacggcggcagctacgccatggactactggggccagggcacaagcgtgaccgtgtctagcgggtccctagacaatgagaagagcaatggaaccattatccatgtgaaagggaaacacctttgtccaagtcccctatttcccggaccttctaagcccttttgggtgctggtggtggttggtggagtcctggcttgctatagcttgctagtaacagtggcctttattattttctgggtgaggagtaagaggagcaggctcctgcacagtgactacatgaacatgactccccgccgccccgggcccacccgcaagcattaccagccctatgccccaccacgcgacttcgcagcctatcgctccctgagagtgaagttcagcaggagcgcagacgcccccgcgtaccagcagggccagaaccagctctataacgagctcaatctaggacgaagagaggagtacgatgttttggacaagaggcgtggccgggaccctgagatggggggaaagccgagaaggaagaaccctcaggaaggcctgtacaatgaactgcagaaagataagatggcggaggcctacagtgagattgggatgaaaggcgagcgccggaggggcaaggggcacgatggcctttaccagggtctcagtacagccaccaaggacacctacgacgcccttcacatgcaggccctgccccctcgct

SEQ ID NO: 101 - protein, 465 aa, Artificial Sequence
  source: /note="Description of Artificial Sequence: Synthetic CD19 CAR DNA sequence"
EQKLISEEDLDIQMTQTTSSLSASLGDRVTISCRASQDISKYLNWYQQKPDGTVKLLIYHTSRLHSGVPSRFSGSGSGTDYSLTISNLEQEDIATYFCQQGNTLPYTFGGGTKLEITGGGGSGGGGSGGGGSEVKLQESGPGLVAPSQSLSVTCTVSGVSLPDYGVSWIRQPPRKGLEWLGVIWGSETTYYNSALKSRLTIIKDNSKSQVFLKMNSLQTDDTAIYYCAKHYYYGGSYAMDYWGQGTSVTVSSGSLDNEKSNGTIIHVKGKHLCPSPLFPGPSKPFWVLVVVGGVLACYSLLVTVAFIIFWVRSKRSRLLHSDYMNMTPRRPGPTRKHYQPYAPPRDFAAYRSLRVKFSRSADAPAYQQGQNQLYNELNLGRREEYDVLDKRRGRDPEMGGKPRRKNPQEGLYNELQKDKMAEAYSEIGMKGERRRGKGHDGLYQGLSTATKDTYDALHMQALPPR

SEQ ID NO: 102 - DNA, 2928 bp, Artificial Sequence
  source: /note="Description of Artificial Sequence: Synthetic CD19 CAR + IL7A_CPT sequence"
gaacagaagctgataagtgaggaggacttggacatccagatgacccagaccaccagcagcctgagcgccagcctgggcgatagagtgaccatcagctgcagagccagccaggacatcagcaagtacctgaactggtatcagcagaaacccgacggcaccgtgaagctgctgatctaccacaccagcagactgcacagcggcgtgcccagcagattttctggcagcggctccggcaccgactacagcctgaccatctccaacctggaacaggaagatatcgctacctacttctgtcagcaaggcaacaccctgccctacaccttcggcggaggcaccaagctggaaatcacaggcggcggaggatctggcggaggcggaagtggcggagggggatctgaagtgaaactgcaggaaagcggccctggcctggtggccccatctcagtctctgagcgtgacctgtaccgtgtccggcgtgtccctgcctgactatggcgtgtcctggatcagacagccccccagaaagggcctggaatggctgggagtgatctggggcagcgagacaacctactacaacagcgccctgaagtcccggctgaccatcatcaaggacaactccaagagccaggtgttcctgaagatgaacagcctgcagaccgacgacaccgccatctactactgcgccaagcactactactacggcggcagctacgccatggactactggggccagggcacaagcgtgaccgtgtctagcgggtccctagacaatgagaagagcaatggaaccattatccatgtgaaagggaaacacctttgtccaagtcccctatttcccggaccttctaagcccttttgggtgctggtggtggttggtggagtcctggcttgctatagcttgctagtaacagtggcctttattattttctgggtgaggagtaagaggagcaggctcctgcacagtgactacatgaacatgactccccgccgccccgggcccacccgcaagcattaccagccctatgccccaccacgcgacttcgcagcctatcgctccctgagagtgaagttcagcaggagcgcagacgcccccgcgtaccagcagggccagaaccagctctataacgagctcaatctaggacgaagagaggagtacgatgttttggacaagaggcgtggccgggaccctgagatggggggaaagccgagaaggaagaaccctcaggaaggcctgtacaatgaactgcagaaagataagatggcggaggcctacagtgagattgggatgaaaggcgagcgccggaggggcaaggggcacgatggcctttaccagggtctcagtacagccaccaaggacacctacgacgcccttcacatgcaggccctgccccctcgccggaagagaagaggcaagcccatccccaacccactgctgggcctggatagcacctccggaagcggagagggcagaggctctctgctgacctgcggcgacgtggaagagaacccagggcccatgctcctgctcgtgacttcacttcttctctgtgaactcccacaccccgcgtttttgcttatccctcatcatcaccatcaccacggcgagagcggctacgcccagaacggcgacctggaggacgccgagctggacgactacagcttcagctgctacagccagctggaggtgaacggcagccagcacagcctgacctgcgccttcgaggaccccgacgtgaacatcaccaacctggagttcgagatctgcggcgccctggtggaggtgaagtgcctgaacttcaggaagctgcaggagatctacttcatcgagaccaagaagttcctgctgatcggcaagagcaacatctgcgtgaaggtgggcgagaagagcctgacctgcaagaagatcgacctgaccaccatcgtgaagcccgaggcccccttcgacctgagcgtggtgtacagggagggcgccaacgacttcgtggtgaccttcaacaccagccacctgcagaagaagtacgtgaaggtgctgatgcacgacgtggcctacaggcaggagaaggacgagaacaagtggacccacgtgaacctgagcagcaccaagctgaccctgctgcagaggaagctgcagcccgccgccatgtacgagatcaaggtgaggagcatccccgaccactacttcaagggcttctggagcgagtggagccccagctactacttcaggacccccgagatcaacaacagcagcggcgagatggaccccatcctgctgacctgccccaccatcagcatcctgagcttcttcagcgtggccctgctggtgatcctggcctgcgtgctgtggaagaagaggatcaagcccatcgtgtggcccagcctgcccgaccacaagaagaccctggagcacctgtgtaagaagcccaggaagaacctgaacgtgagcttcaaccccgagagcttcctggactgccagatccacagggtggacgacatccaggccagggacgaggtggagggcttcctgcaggacaccttcccccagcagctggaggagagcgagaagcagaggctgggcggcgacgtgcagagccccaactgccccagcgaggacgtggtgatcacccccgagagcttcggcagggacagcagcctgacctgcctggccggcaacgtgagcgcctgcgacgcccccatcctgagcagcagcaggagcctggactgcagggagagcggcaagaacggcccccacgtgtaccaggacctgctgctgagcctgggcaccaccaacagcaccctgccaccccccttcagcctgcagagcggcatcctgaccctgaaccccgtggcccagggccagcccatcctgaccagcctgggcagcaaccaggaggaggcctacgtgaccatgagcagcttctaccagaaccag

SEQ ID NO: 103 - protein, 976 aa, Artificial Sequence
  source: /note="Description of Artificial Sequence: Synthetic CD19 CAR + IL7A_CPT sequence"
EQKLISEEDLDIQMTQTTSSLSASLGDRVTISCRASQDISKYLNWYQQKPDGTVKLLIYHTSRLHSGVPSRFSGSGSGTDYSLTISNLEQEDIATYFCQQGNTLPYTFGGGTKLEITGGGGSGGGGSGGGGSEVKLQESGPGLVAPSQSLSVTCTVSGVSLPDYGVSWIRQPPRKGLEWLGVIWGSETTYYNSALKSRLTIIKDNSKSQVFLKMNSLQTDDTAIYYCAKHYYYGGSYAMDYWGQGTSVTVSSGSLDNEKSNGTIIHVKGKHLCPSPLFPGPSKPFWVLVVVGGVLACYSLLVTVAFIIFWVRSKRSRLLHSDYMNMTPRRPGPTRKHYQPYAPPRDFAAYRSLRVKFSRSADAPAYQQGQNQLYNELNLGRREEYDVLDKRRGRDPEMGGKPRRKNPQEGLYNELQKDKMAEAYSEIGMKGERRRGKGHDGLYQGLSTATKDTYDALHMQALPPRRKRRGKPIPNPLLGLDSTSGSGEGRGSLLTCGDVEENPGPMLLLVTSLLLCELPHPAFLLIPHHHHHHGESGYAQNGDLEDAELDDYSFSCYSQLEVNGSQHSLTCAFEDPDVNITNLEFEICGALVEVKCLNFRKLQEIYFIETKKFLLIGKSNICVKVGEKSLTCKKIDLTTIVKPEAPFDLSVVYREGANDFVVTFNTSHLQKKYVKVLMHDVAYRQEKDENKWTHVNLSSTKLTLLQRKLQPAAMYEIKVRSIPDHYFKGFWSEWSPSYYFRTPEINNSSGEMDPILLTCPTISILSFFSVALLVILACVLWKKRIKPIVWPSLPDHKKTLEHLCKKPRKNLNVSFNPESFLDCQIHRVDDIQARDEVEGFLQDTFPQQLEESEKQRLGGDVQSPNCPSEDVVITPESFGRDSSLTCLAGNVSACDAPILSSSRSLDCRESGKNGPHVYQDLLLSLGTTNSTLPPPFSLQSGILTLNPVAQGQPILTSLGSNQEEAYVTMSSFYQNQ

SEQ ID NO: 104 - DNA, 2928 bp, Artificial Sequence
  source: /note="Description of Artificial Sequence: Synthetic CD19 CAR + IL7RaMCP sequence"
gaacagaagctgataagtgaggaggacttggacatccagatgacccagaccaccagcagcctgagcgccagcctgggcgatagagtgaccatcagctgcagagccagccaggacatcagcaagtacctgaactggtatcagcagaaacccgacggcaccgtgaagctgctgatctaccacaccagcagactgcacagcggcgtgcccagcagattttctggcagcggctccggcaccgactacagcctgaccatctccaacctggaacaggaagatatcgctacctacttctgtcagcaaggcaacaccctgccctacaccttcggcggaggcaccaagctggaaatcacaggcggcggaggatctggcggaggcggaagtggcggagggggatctgaagtgaaactgcaggaaagcggccctggcctggtggccccatctcagtctctgagcgtgacctgtaccgtgtccggcgtgtccctgcctgactatggcgtgtcctggatcagacagccccccagaaagggcctggaatggctgggagtgatctggggcagcgagacaacctactacaacagcgccctgaagtcccggctgaccatcatcaaggacaactccaagagccaggtgttcctgaagatgaacagcctgcagaccgacgacaccgccatctactactgcgccaagcactactactacggcggcagctacgccatggactactggggccagggcacaagcgtgaccgtgtctagcgggtccctagacaatgagaagagcaatggaaccattatccatgtgaaagggaaacacctttgtccaagtcccctatttcccggaccttctaagcccttttgggtgctggtggtggttggtggagtcctggcttgctatagcttgctagtaacagtggcctttattattttctgggtgaggagtaagaggagcaggctcctgcacagtgactacatgaacatgactccccgccgccccgggcccacccgcaagcattaccagccctatgccccaccacgcgacttcgcagcctatcgctccctgagagtgaagttcagcaggagcgcagacgcccccgcgtaccagcagggccagaaccagctctataacgagctcaatctaggacgaagagaggagtacgatgttttggacaagaggcgtggccgggaccctgagatggggggaaagccgagaaggaagaaccctcaggaaggcctgtacaatgaactgcagaaagataagatggcggaggcctacagtgagattgggatgaaaggcgagcgccggaggggcaaggggcacgatggcctttaccagggtctcagtacagccaccaaggacacctacgacgcccttcacatgcaggccctgccccctcgccggaagagaagaggcaagcccatccccaacccactgctgggcctggatagcacctccggaagcggagagggcagaggctctctgctgacctgcggcgacgtggaagagaacccagggcccatgctcctgctcgtgacttcacttcttctctgtgaactcccacaccccgcgtttttgcttatccctcatcatcaccatcaccacggcgagagcggctacgcccagaacggcgacctggaggacgccgagctggacgactacagcttcagctgctacagccagctggaggtgaacggcagccagcacagcctgacctgcgccttcgaggaccccgacgtgaacatcaccaacctggagttcgagatctgcggcgccctggtggaggtgaagtgcctgaacttcaggaagctgcaggagatctacttcatcgagaccaagaagttcctgctgatcggcaagagcaacatctgcgtgaaggtgggcgagaagagcctgacctgcaagaagatcgacctgaccaccatcgtgaagcccgaggcccccttcgacctgagcgtggtgtacagggagggcgccaacgacttcgtggtgaccttcaacaccagccacctgcagaagaagtacgtgaaggtgctgatgcacgacgtggcctacaggcaggagaaggacgagaacaagtggacccacgtgaacctgagcagcaccaagctgaccctgctgcagaggaagctgcagcccgccgccatgtacgagatcaaggtgaggagcatccccgaccactacttcaagggcttctggagcgagtggagccccagctactacttcaggacccccgagatcaacaacagcagcggcgagatggaccccatcctgctgatgtgccccaccatcagcatcctgagcttcttcagcgtggccctgctggtgatcctggcctgcgtgctgtggaagaagaggatcaagcccatcgtgtggcccagcctgcccgaccacaagaagaccctggagcacctgtgtaagaagcccaggaagaacctgaacgtgagcttcaaccccgagagcttcctggactgccagatccacagggtggacgacatccaggccagggacgaggtggagggcttcctgcaggacaccttcccccagcagctggaggagagcgagaagcagaggctgggcggcgacgtgcagagccccaactgccccagcgaggacgtggtgatcacccccgagagcttcggcagggacagcagcctgacctgcctggccggcaacgtgagcgcctgcgacgcccccatcctgagcagcagcaggagcctggactgcagggagagcggcaagaacggcccccacgtgtaccaggacctgctgctgagcctgggcaccaccaacagcaccctgccaccccccttcagcctgcagagcggcatcctgaccctgaaccccgtggcccagggccagcccatcctgaccagcctgggcagcaaccaggaggaggcctacgtgaccatgagcagcttctaccagaaccag

SEQ ID NO: 105 - protein, 976 aa, Artificial Sequence
  source: /note="Description of Artificial Sequence: Synthetic CD19 CAR + IL7RaMCP sequence"
EQKLISEEDLDIQMTQTTSSLSASLGDRVTISCRASQDISKYLNWYQQKPDGTVKLLIYHTSRLHSGVPSRFSGSGSGTDYSLTISNLEQEDIATYFCQQGNTLPYTFGGGTKLEITGGGGSGGGGSGGGGSEVKLQESGPGLVAPSQSLSVTCTVSGVSLPDYGVSWIRQPPRKGLEWLGVIWGSETTYYNSALKSRLTIIKDNSKSQVFLKMNSLQTDDTAIYYCAKHYYYGGSYAMDYWGQGTSVTVSSGSLDNEKSNGTIIHVKGKHLCPSPLFPGPSKPFWVLVVVGGVLACYSLLVTVAFIIFWVRSKRSRLLHSDYMNMTPRRPGPTRKHYQPYAPPRDFAAYRSLRVKFSRSADAPAYQQGQNQLYNELNLGRREEYDVLDKRRGRDPEMGGKPRRKNPQEGLYNELQKDKMAEAYSEIGMKGERRRGKGHDGLYQGLSTATKDTYDALHMQALPPRRKRRGKPIPNPLLGLDSTSGSGEGRGSLLTCGDVEENPGPMLLLVTSLLLCELPHPAFLLIPHHHHHHGESGYAQNGDLEDAELDDYSFSCYSQLEVNGSQHSLTCAFEDPDVNITNLEFEICGALVEVKCLNFRKLQEIYFIETKKFLLIGKSNICVKVGEKSLTCKKIDLTTIVKPEAPFDLSVVYREGANDFVVTFNTSHLQKKYVKVLMHDVAYRQEKDENKWTHVNLSSTKLTLLQRKLQPAAMYEIKVRSIPDHYFKGFWSEWSPSYYFRTPEINNSSGEMDPILLMCPTISILSFFSVALLVILACVLWKKRIKPIVWPSLPDHKKTLEHLCKKPRKNLNVSFNPESFLDCQIHRVDDIQARDEVEGFLQDTFPQQLEESEKQRLGGDVQSPNCPSEDVVITPESFGRDSSLTCLAGNVSACDAPILSSSRSLDCRESGKNGPHVYQDLLLSLGTTNSTLPPPFSLQSGILTLNPVAQGQPILTSLGSNQEEAYVTMSSFYQNQ

SEQ ID NO: 106 - DNA, 2931 bp, Artificial Sequence
  source: /note="Description of Artificial Sequence: Synthetic CD19 CAR + IL7RaPPCL sequence"
gaacagaagctgataagtgaggaggacttggacatccagatgacccagaccaccagcagcctgagcgccagcctgggcgatagagtgaccatcagctgcagagccagccaggacatcagcaagtacctgaactggtatcagcagaaacccgacggcaccgtgaagctgctgatctaccacaccagcagactgcacagcggcgtgcccagcagattttctggcagcggctccggcaccgactacagcctgaccatctccaacctggaacaggaagatatcgctacctacttctgtcagcaaggcaacaccctgccctacaccttcggcggaggcaccaagctggaaatcacaggcggcggaggatctggcggaggcggaagtggcggagggggatctgaagtgaaactgcaggaaagcggccctggcctggtggccccatctcagtctctgagcgtgacctgtaccgtgtccggcgtgtccctgcctgactatggcgtgtcctggatcagacagccccccagaaagggcctggaatggctgggagtgatctggggcagcgagacaacctactacaacagcgccctgaagtcccggctgaccatcatcaaggacaactccaagagccaggtgttcctgaagatgaacagcctgcagaccgacgacaccgccatctactactgcgccaagcactactactacggcggcagctacgccatggactactggggccagggcacaagcgtgaccgtgtctagcgggtccctagacaatgagaagagcaatggaaccattatccatgtgaaagggaaacacctttgtccaagtcccctatttcccggaccttctaagcccttttgggtgctggtggtggttggtggagtcctggcttgctatagcttgctagtaacagtggcctttattattttctgggtgaggagtaagaggagcaggctcctgcacagtgactacatgaacatgactccccgccgccccgggcccacccgcaagcattaccagccctatgccccaccacgcgacttcgcagcctatcgctccctgagagtgaagttcagcaggagcgcagacgcccccgcgtaccagcagggccagaaccagctctataacgagctcaatctaggacgaagagaggagtacgatgttttggacaagaggcgtggccgggaccctgagatggggggaaagccgagaaggaagaaccctcaggaaggcctgtacaatgaactgcagaaagataagatggcggaggcctacagtgagattgggatgaaaggcgagcgccggaggggcaaggggcacgatggcctttaccagggtctcagtacagccaccaaggacacctacgacgcccttcacatgcaggccctgccccctcgccggaagagaagaggcaagcccatccccaacccactgctgggcctggatagcacctccggaagcggagagggcagaggctctctgctgacctgcggcgacgtggaagagaacccagggcccatgctcctgctcgtgacttcacttcttctctgtgaactcccacaccccgcgtttttgcttatccctcatcatcaccatcaccacggcgagagcggctacgcccagaacggcgacctggaggacgccgagctggacgactacagcttcagctgctacagccagctggaggtgaacggcagccagcacagcctgacctgcgccttcgaggaccccgacgtgaacatcaccaacctggagttcgagatctgcggcgccctggtggaggtgaagtgcctgaacttcaggaagctgcaggagatctacttcatcgagaccaagaagttcctgctgatcggcaagagcaacatctgcgtgaaggtgggcgagaagagcctgacctgcaagaagatcgacctgaccaccatcgtgaagcccgaggcccccttcgacctgagcgtggtgtacagggagggcgccaacgacttcgtggtgaccttcaacaccagccacctgcagaagaagtacgtgaaggtgctgatgcacgacgtggcctacaggcaggagaaggacgagaacaagtggacccacgtgaacctgagcagcaccaagctgaccctgctgcagaggaagctgcagcccgccgccatgtacgagatcaaggtgaggagcatccccgaccactacttcaagggcttctggagcgagtggagccccagctactacttcaggacccccgagatcaacaacagcagcggcgagatggaccccatcctgctgccaccctgtttaaccatcagcatcctgagcttcttcagcgtggccctgctggtgatcctggcctgcgtgctgtggaagaagaggatcaagcccatcgtgtggcccagcctgcccgaccacaagaagaccctggagcacctgtgtaagaagcccaggaagaacctgaacgtgagcttcaaccccgagagcttcctggactgccagatccacagggtggacgacatccaggccagggacgaggtggagggcttcctgcaggacaccttcccccagcagctggaggagagcgagaagcagaggctgggcggcgacgtgcagagccccaactgccccagcgaggacgtggtgatcacccccgagagcttcggcagggacagcagcctgacctgcctggccggcaacgtgagcgcctgcgacgcccccatcctgagcagcagcaggagcctggactgcagggagagcggcaagaacggcccccacgtgtaccaggacctgctgctgagcctgggcaccaccaacagcaccctgccaccccccttcagcctgcagagcggcatcctgaccctgaaccccgtggcccagggccagcccatcctgaccagcctgggcagcaaccaggaggaggcctacgtgaccatgagcagcttctaccagaaccag

SEQ ID NO: 107 - protein, 977 aa, Artificial Sequence
  source: /note="Description of Artificial Sequence: Synthetic CD19 CAR + IL7RaPPCL sequence"
EQKLISEEDLDIQMTQTTSSLSASLGDRVTISCRASQDISKYLNWYQQKPDGTVKLLIYHTSRLHSGVPSRFSGSGSGTDYSLTISNLEQEDIATYFCQQGNTLPYTFGGGTKLEITGGGGSGGGGSGGGGSEVKLQESGPGLVAPSQSLSVTCTVSGVSLPDYGVSWIRQPPRKGLEWLGVIWGSETTYYNSALKSRLTIIKDNSKSQVFLKMNSLQTDDTAIYYCAKHYYYGGSYAMDYWGQGTSVTVSSGSLDNEKSNGTIIHVKGKHLCPSPLFPGPSKPFWVLVVVGGVLACYSLLVTVAFIIFWVRSKRSRLLHSDYMNMTPRRPGPTRKHYQPYAPPRDFAAYRSLRVKFSRSADAPAYQQGQNQLYNELNLGRREEYDVLDKRRGRDPEMGGKPRRKNPQEGLYNELQKDKMAEAYSEIGMKGERRRGKGHDGLYQGLSTATKDTYDALHMQALPPRRKRRGKPIPNPLLGLDSTSGSGEGRGSLLTCGDVEENPGPMLLLVTSLLLCELPHPAFLLIPHHHHHHGESGYAQNGDLEDAELDDYSFSCYSQLEVNGSQHSLTCAFEDPDVNITNLEFEICGALVEVKCLNFRKLQEIYFIETKKFLLIGKSNICVKVGEKSLTCKKIDLTTIVKPEAPFDLSVVYREGANDFVVTFNTSHLQKKYVKVLMHDVAYRQEKDENKWTHVNLSSTKLTLLQRKLQPAAMYEIKVRSIPDHYFKGFWSEWSPSYYFRTPEINNSSGEMDPILLPPCLTISILSFFSVALLVILACVLWKKRIKPIVWPSLPDHKKTLEHLCKKPRKNLNVSFNPESFLDCQIHRVDDIQARDEVEGFLQDTFPQQLEESEKQRLGGDVQSPNCPSEDVVITPESFGRDSSLTCLAGNVSACDAPILSSSRSLDCRESGKNGPHVYQDLLLSLGTTNSTLPPPFSLQSGILTLNPVAQGQPILTSLGSNQEEAYVTMSSFYQNQ

SEQ ID NO: 108 - DNA, 1419 bp, Artificial Sequence
  source: /note="Description of Artificial Sequence: Synthetic GPC3 CAR sequence"
gatatcgtgatgacccagagccccgactctttagctgtgtctttaggagagagggccacaatcaactgcaagagcagccagagcctcctctacagcagcaaccagaagaactatttagcttggtaccagcaaaagcccggccagccccccaagctgctgatctactgggccagcagcagagagagcggcgtgcccgatagattcagcggaagcggctccggcacagatttcaccctcaccattagctctttacaagctgaggacgtggccgtgtactactgccagcagtactacaactaccctttaaccttcggccaaggtaccaagctggagatcaagggctccacatccggatccggcaagcccggtagcggagaaggcagcacaaagggagaggtgcagctggtggagagcggaggcggactggtccagcccggtggatctttaaggctgtcttgtgccgccagcggctttacctttaacaagaacgctatgaactgggtgaggcaagctcccggtaagggtttagagtgggtgggtcgtattcgtaataagaccaacaactacgccacctactatgccgactccgtgaaggctcgtttcaccatctctcgtgacgacagcaagaacagcctctatttacagatgaactctttaaagaccgaggacaccgccgtgtactattgcgtggctggcaactccttcgcctactggggccaaggcactttagtgaccgtgagctccgggtccaccacgacgccagcgccgcgaccaccaacaccggcgcccaccatcgcgtcgcagcccctgtccctgcgcccagaggcgtgccggccagcggcggggggcgcagtgcacacgagggggctggacttcgcctgtgatatctacatctgggcgcccttggccgggacttgtggggtccttctcctgtcactggttatcaccctttactgcaaacggggcagaaagaaactcctgtatatattcaaacaaccatttatgagaccagtacaaactactcaagaggaagatggctgtagctgccgatttccagaagaagaagaaggaggatgtgaactgagagtgaagttcagcaggagcgcagacgcccccgcgtaccagcagggccagaaccagctctataacgagctcaatctaggacgaagagaggagtacgatgttttggacaagaggcgtggccgggaccctgagatggggggaaagccgagaaggaagaaccctcaggaaggcctgtacaatgaactgcagaaagataagatggcggaggcctacagtgagattgggatgaaaggcgagcgccggaggggcaaggggcacgatggcctttaccagggtctcagtacagccaccaaggacacctacgacgcccttcacatgcaggccctgccccctcgc

SEQ ID NO: 109 - protein, 473 aa, Artificial Sequence
  source: /note="Description of Artificial Sequence: Synthetic GPC3 CAR sequence"
DIVMTQSPDSLAVSLGERATINCKSSQSLLYSSNQKNYLAWYQQKPGQPPKLLIYWASSRESGVPDRFSGSGSGTDFTLTISSLQAEDVAVYYCQQYYNYPLTFGQGTKLEIKGSTSGSGKPGSGEGSTKGEVQLVESGGGLVQPGGSLRLSCAASGFTFNKNAMNWVRQAPGKGLEWVGRIRNKTNNYATYYADSVKARFTISRDDSKNSLYLQMNSLKTEDTAVYYCVAGNSFAYWGQGTLVTVSSGSTTTPAPRPPTPAPTIASQPLSLRPEACRPAAGGAVHTRGLDFACDIYIWAPLAGTCGVLLLSLVITLYCKRGRKKLLYIFKQPFMRPVQTTQEEDGCSCRFPEEEEGGCELRVKFSRSADAPAYQQGQNQLYNELNLGRREEYDVLDKRRGRDPEMGGKPRRKNPQEGLYNELQKDKMAEAYSEIGMKGERRRGKGHDGLYQGLSTATKDTYDALHMQALPPR

SEQ ID NO: 110 - DNA, 2895 bp, Artificial Sequence
  source: /note="Description of Artificial Sequence: Synthetic GPC3 CAR + IL7aCPT sequence"
gatatcgtgatgacccagagccccgactctttagctgtgtctttaggagagagggccacaatcaactgcaagagcagccagagcctcctctacagcagcaaccagaagaactatttagcttggtaccagcaaaagcccggccagccccccaagctgctgatctactgggccagcagcagagagagcggcgtgcccgatagattcagcggaagcggctccggcacagatttcaccctcaccattagctctttacaagctgaggacgtggccgtgtactactgccagcagtactacaactaccctttaaccttcggccaaggtaccaagctggagatcaagggctccacatccggatccggcaagcccggtagcggagaaggcagcacaaagggagaggtgcagctggtggagagcggaggcggactggtccagcccggtggatctttaaggctgtcttgtgccgccagcggctttacctttaacaagaacgctatgaactgggtgaggcaagctcccggtaagggtttagagtgggtgggtcgtattcgtaataagaccaacaactacgccacctactatgccgactccgtgaaggctcgtttcaccatctctcgtgacgacagcaagaacagcctctatttacagatgaactctttaaagaccgaggacaccgccgtgtactattgcgtggctggcaactccttcgcctactggggccaaggcactttagtgaccgtgagctccgggtccaccacgacgccagcgccgcgaccaccaacaccggcgcccaccatcgcgtcgcagcccctgtccctgcgcccagaggcgtgccggccagcggcggggggcgcagtgcacacgagggggctggacttcgcctgtgatatctacatctgggcgcccttggccgggacttgtggggtccttctcctgtcactggttatcaccctttactgcaaacggggcagaaagaaactcctgtatatattcaaacaaccatttatgagaccagtacaaactactcaagaggaagatggctgtagctgccgatttccagaagaagaagaaggaggatgtgaactgagagtgaagttcagcaggagcgcagacgcccccgcgtaccagcagggccagaaccagctctataacgagctcaatctaggacgaagagaggagtacgatgttttggacaagaggcgtggccgggaccctgagatggggggaaagccgagaaggaagaaccctcaggaaggcctgtacaatgaactgcagaaagataagatggcggaggcctacagtgagattgggatgaaaggcgagcgccggaggggcaaggggcacgatggcctttaccagggtctcagtacagccaccaaggacacctacgacgcccttcacatgcaggccctgccccctcgcgggtccggagagggcagaggctctctgctgacctgcggcgacgtggaagagaacccagggcccatgctcctgctcgtgacttcacttcttctctgtgaactcccacaccccgcgtttttgcttatccctcatcatcaccatcaccacggcgagagcggctacgcccagaacggcgacctggaggacgccgagctggacgactacagcttcagctgctacagccagctggaggtgaacggcagccagcacagcctgacctgcgccttcgaggaccccgacgtgaacatcaccaacctggagttcgagatctgcggcgccctggtggaggtgaagtgcctgaacttcaggaagctgcaggagatctacttcatcgagaccaagaagttcctgctgatcggcaagagcaacatctgcgtgaaggtgggcgagaagagcctgacctgcaagaagatcgacctgaccaccatcgtgaagcccgaggcccccttcgacctgagcgtggtgtacagggagggcgccaacgacttcgtggtgaccttcaacaccagccacctgcagaagaagtacgtgaaggtgctgatgcacgacgtggcctacaggcaggagaaggacgagaacaagtggacccacgtgaacctgagcagcaccaagctgaccctgctgcagaggaagctgcagcccgccgccatgtacgagatcaaggtgaggagcatccccgaccactacttcaagggcttctggagcgagtggagccccagctactacttcaggacccccgagatcaacaacagcagcggcgagatggaccccatcctgctgacctgccccaccatcagcatcctgagcttcttcagcgtggccctgctggtgatcctggcctgcgtgctgtggaagaagaggatcaagcccatcgtgtggcccagcctgcccgaccacaagaagaccctggagcacctgtgtaagaagcccaggaagaacctgaacgtgagcttcaaccccgagagcttcctggactgccagatccacagggtggacgacatccaggccagggacgaggtggagggcttcctgcaggacaccttcccccagcagctggaggagagcgagaagcagaggctgggcggcgacgtgcagagccccaactgccccagcgaggacgtggtgatcacccccgagagcttcggcagggacagcagcctgacctgcctggccggcaacgtgagcgcctgcgacgcccccatcctgagcagcagcaggagcctggactgcagggagagcggcaagaacggcccccacgtgtaccaggacctgctgctgagcctgggcaccaccaacagcaccctgccaccccccttcagcctgcagagcggcatcctgaccctgaaccccgtggcccagggccagcccatcctgaccagcctgggcagcaaccaggaggaggcctacgtgaccatgagcagcttctaccagaaccag

SEQ ID NO: 111 - protein, 965 aa, Artificial Sequence
  source: /note="Description of Artificial Sequence: Synthetic GPC3 CAR + IL7aCPT sequence"
DIVMTQSPDSLAVSLGERATINCKSSQSLLYSSNQKNYLAWYQQKPGQPPKLLIYWASSRESGVPDRFSGSGSGTDFTLTISSLQAEDVAVYYCQQYYNYPLTFGQGTKLEIKGSTSGSGKPGSGEGSTKGEVQLVESGGGLVQPGGSLRLSCAASGFTFNKNAMNWVRQAPGKGLEWVGRIRNKTNNYATYYADSVKARFTISRDDSKNSLYLQMNSLKTEDTAVYYCVAGNSFAYWGQGTLVTVSSGSTTTPAPRPPTPAPTIASQPLSLRPEACRPAAGGAVHTRGLDFACDIYIWAPLAGTCGVLLLSLVITLYCKRGRKKLLYIFKQPFMRPVQTTQEEDGCSCRFPEEEEGGCELRVKFSRSADAPAYQQGQNQLYNELNLGRREEYDVLDKRRGRDPEMGGKPRRKNPQEGLYNELQKDKMAEAYSEIGMKGERRRGKGHDGLYQGLSTATKDTYDALHMQALPPRGSGEGRGSLLTCGDVEENPGPMLLLVTSLLLCELPHPAFLLIPHHHHHHGESGYAQNGDLEDAELDDYSFSCYSQLEVNGSQHSLTCAFEDPDVNITNLEFEICGALVEVKCLNFRKLQEIYFIETKKFLLIGKSNICVKVGEKSLTCKKIDLTTIVKPEAPFDLSVVYREGANDFVVTFNTSHLQKKYVKVLMHDVAYRQEKDENKWTHVNLSSTKLTLLQRKLQPAAMYEIKVRSIPDHYFKGFWSEWSPSYYFRTPEINNSSGEMDPILLTCPTISILSFFSVALLVILACVLWKKRIKPIVWPSLPDHKKTLEHLCKKPRKNLNVSFNPESFLDCQIHRVDDIQARDEVEGFLQDTFPQQLEESEKQRLGGDVQSPNCPSEDVVITPESFGRDSSLTCLAGNVSACDAPILSSSRSLDCRESGKNGPHVYQDLLLSLGTTNSTLPPPFSLQSGILTLNPVAQGQPILTSLGSNQEEAYVTMSSFYQNQ